European Patent Specification EP 3 481 861 B1, published July 31, 2024. Title: SEQUENTIAL GENE EDITING IN PRIMARY IMMUNE CELLS. Applicant: Cellectis. The sequence listing filed with the application follows.

SEQUENCE LISTING (12 sequences)

SEQ ID NO: 1 - protein, 925 aa, artificial sequence
  TRAC TALEN Left
MGDPKKKRKVIDIADLRTLGYSQQQQEKIKPKVRSTVAQHHEALVGHGFTHAHIVALSQHPAALGTVAVKYQDMIAALPEATHEAIVGVGKQWSGARALEALLTVAGELRGPPLQLDTGQLLKIAKRGGVTAVEAVHAWRNALTGAPLNLTPQQVVAIASNGGGKQALETVQRLLPVLCQAHGLTPQQVVAIASNNGGKQALETVQRLLPVLCQAHGLTPQQVVAIASNGGGKQALETVQRLLPVLCQAHGLTPEQVVAIASHDGGKQALETVQRLLPVLCQAHGLTPEQVVAIASHDGGKQALETVQRLLPVLCQAHGLTPEQVVAIASHDGGKQALETVQRLLPVLCQAHGLTPEQVVAIASNIGGKQALETVQALLPVLCQAHGLTPEQVVAIASHDGGKQALETVQRLLPVLCQAHGLTPEQVVAIASNIGGKQALETVQALLPVLCQAHGLTPQQVVAIASNNGGKQALETVQRLLPVLCQAHGLTPEQVVAIASNIGGKQALETVQALLPVLCQAHGLTPQQVVAIASNGGGKQALETVQRLLPVLCQAHGLTPEQVVAIASNIGGKQALETVQALLPVLCQAHGLTPQQVVAIASNGGGKQALETVQRLLPVLCQAHGLTPEQVVAIASHDGGKQALETVQRLLPVLCQAHGLTPQQVVAIASNGGGRPALESIVAQLSRPDPALAALTNDHLVALACLGGRPALDAVKKGLGDPISRSQLVKSELEEKKSELRHKLKYVPHEYIELIEIARNSTQDRILEMKVMEFFMKVYGYRGKHLGGSRKPDGAIYTVGSPIDYGVIVDTKAYSGGYNLPIGQADEMQRYVEENQTRNKHINPNEWWKVYPSSVTEFKFLFVSGHFKGNYKAQLTRLNHITNCNGAVLSVEELLIGGEMIKAGTLTLEEVRRKFNNGEINFAAD

SEQ ID NO: 2 - protein, 925 aa, artificial sequence
  TRAC TALEN Right
MGDPKKKRKVIDIADLRTLGYSQQQQEKIKPKVRSTVAQHHEALVGHGFTHAHIVALSQHPAALGTVAVKYQDMIAALPEATHEAIVGVGKQWSGARALEALLTVAGELRGPPLQLDTGQLLKIAKRGGVTAVEAVHAWRNALTGAPLNLTPEQVVAIASHDGGKQALETVQRLLPVLCQAHGLTPQQVVAIASNGGGKQALETVQRLLPVLCQAHGLTPEQVVAIASHDGGKQALETVQRLLPVLCQAHGLTPEQVVAIASNIGGKQALETVQALLPVLCQAHGLTPQQVVAIASNNGGKQALETVQRLLPVLCQAHGLTPEQVVAIASHDGGKQALETVQRLLPVLCQAHGLTPQQVVAIASNGGGKQALETVQRLLPVLCQAHGLTPQQVVAIASNNGGKQALETVQRLLPVLCQAHGLTPQQVVAIASNNGGKQALETVQRLLPVLCQAHGLTPQQVVAIASNGGGKQALETVQRLLPVLCQAHGLTPEQVVAIASNIGGKQALETVQALLPVLCQAHGLTPEQVVAIASHDGGKQALETVQRLLPVLCQAHGLTPEQVVAIASNIGGKQALETVQALLPVLCQAHGLTPEQVVAIASHDGGKQALETVQRLLPVLCQAHGLTPQQVVAIASNNGGKQALETVQRLLPVLCQAHGLTPQQVVAIASNGGGRPALESIVAQLSRPDPALAALTNDHLVALACLGGRPALDAVKKGLGDPISRSQLVKSELEEKKSELRHKLKYVPHEYIELIEIARNSTQDRILEMKVMEFFMKVYGYRGKHLGGSRKPDGAIYTVGSPIDYGVIVDTKAYSGGYNLPIGQADEMQRYVEENQTRNKHINPNEWWKVYPSSVTEFKFLFVSGHFKGNYKAQLTRLNHITNCNGAVLSVEELLIGGEMIKAGTLTLEEVRRKFNNGEINFAAD

SEQ ID NO: 3 - protein, 925 aa, artificial sequence
  CD52 TALEN Left
MGDPKKKRKVIDIADLRTLGYSQQQQEKIKPKVRSTVAQHHEALVGHGFTHAHIVALSQHPAALGTVAVKYQDMIAALPEATHEAIVGVGKQWSGARALEALLTVAGELRGPPLQLDTGQLLKIAKRGGVTAVEAVHAWRNALTGAPLNLTPQQVVAIASNGGGKQALETVQRLLPVLCQAHGLTPEQVVAIASHDGGKQALETVQRLLPVLCQAHGLTPEQVVAIASHDGGKQALETVQRLLPVLCQAHGLTPQQVVAIASNGGGKQALETVQRLLPVLCQAHGLTPEQVVAIASHDGGKQALETVQRLLPVLCQAHGLTPEQVVAIASHDGGKQALETVQRLLPVLCQAHGLTPQQVVAIASNGGGKQALETVQRLLPVLCQAHGLTPEQVVAIASNIGGKQALETVQALLPVLCQAHGLTPEQVVAIASHDGGKQALETVQRLLPVLCQAHGLTPQQVVAIASNGGGKQALETVQRLLPVLCQAHGLTPEQVVAIASHDGGKQALETVQRLLPVLCQAHGLTPEQVVAIASNIGGKQALETVQALLPVLCQAHGLTPEQVVAIASHDGGKQALETVQRLLPVLCQAHGLTPEQVVAIASHDGGKQALETVQRLLPVLCQAHGLTPEQVVAIASNIGGKQALETVQALLPVLCQAHGLTPQQVVAIASNGGGRPALESIVAQLSRPDPALAALTNDHLVALACLGGRPALDAVKKGLGDPISRSQLVKSELEEKKSELRHKLKYVPHEYIELIEIARNSTQDRILEMKVMEFFMKVYGYRGKHLGGSRKPDGAIYTVGSPIDYGVIVDTKAYSGGYNLPIGQADEMQRYVEENQTRNKHINPNEWWKVYPSSVTEFKFLFVSGHFKGNYKAQLTRLNHITNCNGAVLSVEELLIGGEMIKAGTLTLEEVRRKFNNGEINFAAD

SEQ ID NO: 4 - protein, 925 aa, artificial sequence
  CD52 TALEN Right
MGDPKKKRKVIDIADLRTLGYSQQQQEKIKPKVRSTVAQHHEALVGHGFTHAHIVALSQHPAALGTVAVKYQDMIAALPEATHEAIVGVGKQWSGARALEALLTVAGELRGPPLQLDTGQLLKIAKRGGVTAVEAVHAWRNALTGAPLNLTPQQVVAIASNGGGKQALETVQRLLPVLCQAHGLTPQQVVAIASNNGGKQALETVQRLLPVLCQAHGLTPEQVVAIASHDGGKQALETVQRLLPVLCQAHGLTPQQVVAIASNGGGKQALETVQRLLPVLCQAHGLTPEQVVAIASHDGGKQALETVQRLLPVLCQAHGLTPQQVVAIASNGGGKQALETVQRLLPVLCQAHGLTPQQVVAIASNGGGKQALETVQRLLPVLCQAHGLTPEQVVAIASNIGGKQALETVQALLPVLCQAHGLTPEQVVAIASHDGGKQALETVQRLLPVLCQAHGLTPEQVVAIASHDGGKQALETVQRLLPVLCQAHGLTPQQVVAIASNGGGKQALETVQRLLPVLCQAHGLTPQQVVAIASNNGGKQALETVQRLLPVLCQAHGLTPQQVVAIASNGGGKQALETVQRLLPVLCQAHGLTPEQVVAIASNIGGKQALETVQALLPVLCQAHGLTPEQVVAIASHDGGKQALETVQRLLPVLCQAHGLTPQQVVAIASNGGGRPALESIVAQLSRPDPALAALTNDHLVALACLGGRPALDAVKKGLGDPISRSQLVKSELEEKKSELRHKLKYVPHEYIELIEIARNSTQDRILEMKVMEFFMKVYGYRGKHLGGSRKPDGAIYTVGSPIDYGVIVDTKAYSGGYNLPIGQADEMQRYVEENQTRNKHINPNEWWKVYPSSVTEFKFLFVSGHFKGNYKAQLTRLNHITNCNGAVLSVEELLIGGEMIKAGTLTLEEVRRKFNNGEINFAAD

SEQ ID NO: 5 - protein, 925 aa, artificial sequence
  PD-1 TALEN Left
MGDPKKKRKVIDIADLRTLGYSQQQQEKIKPKVRSTVAQHHEALVGHGFTHAHIVALSQHPAALGTVAVKYQDMIAALPEATHEAIVGVGKQWSGARALEALLTVAGELRGPPLQLDTGQLLKIAKRGGVTAVEAVHAWRNALTGAPLNLTPEQVVAIASGNGGKQALETVQALLPVLCQAHGLTPEQVVAIASHDGGKQALETVQRLLPVLCQAHGLTPEQVVAIASHDGGKQALETVQRLLPVLCQAHGLTPQQVVAIASNGGGKQALETVQRLLPVLCQAHGLTPEQVVAIASHDGGKQALETVQRLLPVLCQAHGLTPQQVVAIASNGGGKQALETVQRLLPVLCQAHGLTPQQVVAIASNNGGKQALETVQRLLPVLCQAHGLTPQQVVAIASNGGGKQALETVQRLLPVLCQAHGLTPQQVVAIASGRGGKQALETVQRLLPVLCQAHGLTPQQVVAIASNNGGKQALETVQRLLPVLCQAHGLTPQQVVAIASNNGGKQALETVQRLLPVLCQAHGLTPQQVVAIASNNGGKQALETVQRLLPVLCQAHGLTPEQVVAIASHDGGKQALETVQRLLPVLCQAHGLTPEQVVAIASHDGGKQALETVQRLLPVLCQAHGLTPEQVVAIASNIGGKQALETVQALLPVLCQAHGLTPQQVVAIASNGGGRPALESIVAQLSRPDPALAALTNDHLVALACLGGRPALDAVKKGLGDPISRSQLVKSELEEKKSELRHKLKYVPHEYIELIEIARNSTQDRILEMKVMEFFMKVYGYRGKHLGGSRKPDGAIYTVGSPIDYGVIVDTKAYSGGYNLPIGQADEMQRYVEENQTRNKHINPNEWWKVYPSSVTEFKFLFVSGHFKGNYKAQLTRLNHITNCNGAVLSVEELLIGGEMIKAGTLTLEEVRRKFNNGEINFAAD

SEQ ID NO: 6 - protein, 924 aa, artificial sequence
  PD-1 TALEN Right
MGDPKKKRKVIDIADLRTLGYSQQQQEKIKPKVRSTVAQHHEALVGHGFTHAHIVALSQHPAALGTVAVKYQDMIAALPEATHEAIVGVGKQWSGARALEALLTVAGELRGPPLQLDTGQLLKIAKRGGVTAVEAVHAWRNALTGAPLNLTPEQVVAIASHDGGKQALETVQRLLPVLCQAHGLTPQQVVAIASNGGGKQALETVQRLLPVLCQAHGLTPEQVVAIASHDGGKQALETVQRLLPVLCQAHGLTPQQVVAIASNGGGKQALETVQRLLPVLCQAHGLTPQQVVAIASNGGGKQALETVQRLLPVLCQAHGLTPQQVVAIASNGGGKQALETVQRLLPVLCQAHGLTPQQVVAIASNNGGKQALETVQRLLPVLCQAHGLTPEQVVAIASNIGGKQALETVQALLPVLCQAHGLTPQQVVAIASNGGGKQALETVQRLLPVLCQAHGLTPEQVVAIASHDGGKQALETVQRLLPVLCQAHGLTPQQVVAIASNGGGKQALETVQRLLPVLCQAHGLTPQQVVAIASNNGGKQALETVQRLLPVLCQAHGLTPEQVVAIASNGGKQALETVQRLLPVLCQAHGLTPQQVVAIASNNGGKQALETVQRLLPVLCQAHGLTPEQVVAIASHDGGKQALETVQRLLPVLCQAHGLTPQQVVAIASNGGGRPALESIVAQLSRPDPALAALTNDHLVALACLGGRPALDAVKKGLGDPISRSQLVKSELEEKKSELRHKLKYVPHEYIELIEIARNSTQDRILEMKVMEFFMKVYGYRGKHLGGSRKPDGAIYTVGSPIDYGVIVDTKAYSGGYNLPIGQADEMQRYVEENQTRNKHINPNEWWKVYPSSVTEFKFLFVSGHFKGNYKAQLTRLNHITNCNGAVLSVEELLIGGEMIKAGTLTLEEVRRKFNNGEINFAAD

SEQ ID NO: 7 - protein, 925 aa, artificial sequence
  CD38 TALEN Left
MGDPKKKRKVIDIADLRTLGYSQQQQEKIKPKVRSTVAQHHEALVGHGFTHAHIVALSQHPAALGTVAVKYQDMIAALPEATHEAIVGVGKQWSGARALEALLTVAGELRGPPLQLDTGQLLKIAKRGGVTAVEAVHAWRNALTGAPLNLTPQQVVAIASNNGGKQALETVQRLLPVLCQAHGLTPEQVVAIASHDGGKQALETVQRLLPVLCQAHGLTPQQVVAIASNNGGKQALETVQRLLPVLCQAHGLTPEQVVAIASNIGGKQALETVQALLPVLCQAHGLTPQQVVAIASNNGGKQALETVQRLLPVLCQAHGLTPQQVVAIASNGGGKQALETVQRLLPVLCQAHGLTPQQVVAIASNGGGKQALETVQRLLPVLCQAHGLTPEQVVAIASHDGGKQALETVQRLLPVLCQAHGLTPEQVVAIASNIGGKQALETVQALLPVLCQAHGLTPQQVVAIASNNGGKQALETVQRLLPVLCQAHGLTPEQVVAIASHDGGKQALETVQRLLPVLCQAHGLTPEQVVAIASHDGGKQALETVQRLLPVLCQAHGLTPEQVVAIASHDGGKQALETVQRLLPVLCQAHGLTPQQVVAIASNNGGKQALETVQRLLPVLCQAHGLTPQQVVAIASNNGGKQALETVQRLLPVLCQAHGLTPQQVVAIASNGGGRPALESIVAQLSRPDPALAALTNDHLVALACLGGRPALDAVKKGLGDPISRSQLVKSELEEKKSELRHKLKYVPHEYIELIEIARNSTQDRILEMKVMEFFMKVYGYRGKHLGGSRKPDGAIYTVGSPIDYGVIVDTKAYSGGYNLPIGQADEMQRYVEENQTRNKHINPNEWWKVYPSSVTEFKFLFVSGHFKGNYKAQLTRLNHITNCNGAVLSVEELLIGGEMIKAGTLTLEEVRRKFNNGEINFAAD

SEQ ID NO: 8 - protein, 925 aa, artificial sequence
  CD38 TALEN Right
MGDPKKKRKVIDIADLRTLGYSQQQQEKIKPKVRSTVAQHHEALVGHGFTHAHIVALSQHPAALGTVAVKYQDMIAALPEATHEAIVGVGKQWSGARALEALLTVAGELRGPPLQLDTGQLLKIAKRGGVTAVEAVHAWRNALTGAPLNLTPEQVVAIASNIGGKQALETVQALLPVLCQAHGLTPQQVVAIASNNGGKQALETVQRLLPVLCQAHGLTPEQVVAIASNIGGKQALETVQALLPVLCQAHGLTPQQVVAIASNNGGKQALETVQRLLPVLCQAHGLTPEQVVAIASNIGGKQALETVQALLPVLCQAHGLTPQQVVAIASNNGGKQALETVQRLLPVLCQAHGLTPEQVVAIASHDGGKQALETVQRLLPVLCQAHGLTPEQVVAIASHDGGKQALETVQRLLPVLCQAHGLTPQQVVAIASNNGGKQALETVQRLLPVLCQAHGLTPQQVVAIASNNGGKQALETVQRLLPVLCQAHGLTPEQVVAIASHDGGKQALETVQRLLPVLCQAHGLTPEQVVAIASNIGGKQALETVQALLPVLCQAHGLTPQQVVAIASNNGGKQALETVQRLLPVLCQAHGLTPEQVVAIASHDGGKQALETVQRLLPVLCQAHGLTPEQVVAIASNIGGKQALETVQALLPVLCQAHGLTPQQVVAIASNGGGRPALESIVAQLSRPDPALAALTNDHLVALACLGGRPALDAVKKGLGDPISRSQLVKSELEEKKSELRHKLKYVPHEYIELIEIARNSTQDRILEMKVMEFFMKVYGYRGKHLGGSRKPDGAIYTVGSPIDYGVIVDTKAYSGGYNLPIGQADEMQRYVEENQTRNKHINPNEWWKVYPSSVTEFKFLFVSGHFKGNYKAQLTRLNHITNCNGAVLSVEELLIGGEMIKAGTLTLEEVRRKFNNGEINFAAD

SEQ ID NO: 9 - protein, 925 aa, artificial sequence
  PD-1 TALEN Left 2
MGDPKKKRKVIDIADLRTLGYSQQQQEKIKPKVRSTVAQHHEALVGHGFTHAHIVALSQHPAALGTVAVKYQDMIAALPEATHEAIVGVGKQWSGARALEALLTVAGELRGPPLQLDTGQLLKIAKRGGVTAVEAVHAWRNALTGAPLNLTPEQVVAIASKLGGKQALETVQALLPVLCQAHGLTPEQVVAIASHDGGKQALETVQRLLPVLCQAHGLTPEQVVAIASHDGGKQALETVQRLLPVLCQAHGLTPQQVVAIASNGGGKQALETVQRLLPVLCQAHGLTPEQVVAIASHDGGKQALETVQRLLPVLCQAHGLTPQQVVAIASNGGGKQALETVQRLLPVLCQAHGLTPQQVVAIASYKGGKQALETVQRLLPVLCQAHGLTPQQVVAIASNGGGKQALETVQRLLPVLCQAHGLTPQQVVAIASNNGGKQALETVQRLLPVLCQAHGLTPQQVVAIASNNGGKQALETVQRLLPVLCQAHGLTPQQVVAIASNNGGKQALETVQRLLPVLCQAHGLTPQQVVAIASNNGGKQALETVQRLLPVLCQAHGLTPEQVVAIASHDGGKQALETVQRLLPVLCQAHGLTPEQVVAIASHDGGKQALETVQRLLPVLCQAHGLTPEQVVAIASNIGGKQALETVQALLPVLCQAHGLTPQQVVAIASNGGGRPALESIVAQLSRPDPALAALTNDHLVALACLGGRPALDAVKKGLGDPISRSQLVKSELEEKKSELRHKLKYVPHEYIELIEIARNSTQDRILEMKVMEFFMKVYGYRGKHLGGSRKPDGAIYTVGSPIDYGVIVDTKAYSGGYNLPIGQADEMQRYVEENQTRNKHINPNEWWKVYPSSVTEFKFLFVSGHFKGNYKAQLTRLNHITNCNGAVLSVEELLIGGEMIKAGTLTLEEVRRKFNNGEINFAAD

SEQ ID NO: 10 - protein, 925 aa, artificial sequence
  B2M TALEN left
MGDPKKKRKVIDIADLRTLGYSQQQQEKIKPKVRSTVAQHHEALVGHGFTHAHIVALSQHPAALGTVAVKYQDMIAALPEATHEAIVGVGKQWSGARALEALLTVAGELRGPPLQLDTGQLLKIAKRGGVTAVEAVHAWRNALTGAPLNLTPQQVVAIASNNGGKQALETVQRLLPVLCQAHGLTPQQVVAIASNNGGKQALETVQRLLPVLCQAHGLTPEQVVAIASHDGGKQALETVQRLLPVLCQAHGLTPEQVVAIASHDGGKQALETVQRLLPVLCQAHGLTPQQVVAIASNGGGKQALETVQRLLPVLCQAHGLTPQQVVAIASNGGGKQALETVQRLLPVLCQAHGLTPEQVVAIASNIGGKQALETVQALLPVLCQAHGLTPQQVVAIASNNGGKQALETVQRLLPVLCQAHGLTPEQVVAIASHDGGKQALETVQRLLPVLCQAHGLTPQQVVAIASNGGGKQALETVQRLLPVLCQAHGLTPQQVVAIASNNGGKQALETVQRLLPVLCQAHGLTPQQVVAIASNGGGKQALETVQRLLPVLCQAHGLTPQQVVAIASNNGGKQALETVQRLLPVLCQAHGLTPEQVVAIASHDGGKQALETVQRLLPVLCQAHGLTPQQVVAIASNGGGKQALETVQRLLPVLCQAHGLTPQQVVAIASNGGGRPALESIVAQLSRPDPALAALTNDHLVALACLGGRPALDAVKKGLGDPISRSQLVKSELEEKKSELRHKLKYVPHEYIELIEIARNSTQDRILEMKVMEFFMKVYGYRGKHLGGSRKPDGAIYTVGSPIDYGVIVDTKAYSGGYNLPIGQADEMQRYVEENQTRNKHINPNEWWKVYPSSVTEFKFLFVSGHFKGNYKAQLTRLNHITNCNGAVLSVEELLIGGEMIKAGTLTLEEVRRKFNNGEINFAAD

SEQ ID NO: 11 - protein, 925 aa, artificial sequence
  B2M TALEN right
MGDPKKKRKVIDIADLRTLGYSQQQQEKIKPKVRSTVAQHHEALVGHGFTHAHIVALSQHPAALGTVAVKYQDMIAALPEATHEAIVGVGKQWSGARALEALLTVAGELRGPPLQLDTGQLLKIAKRGGVTAVEAVHAWRNALTGAPLNLTPEQVVAIASNIGGKQALETVQALLPVLCQAHGLTPQQVVAIASNNGGKQALETVQRLLPVLCQAHGLTPEQVVAIASHDGGKQALETVQRLLPVLCQAHGLTPEQVVAIASHDGGKQALETVQRLLPVLCQAHGLTPQQVVAIASNGGGKQALETVQRLLPVLCQAHGLTPEQVVAIASHDGGKQALETVQRLLPVLCQAHGLTPEQVVAIASHDGGKQALETVQRLLPVLCQAHGLTPEQVVAIASNIGGKQALETVQALLPVLCQAHGLTPQQVVAIASNNGGKQALETVQRLLPVLCQAHGLTPQQVVAIASNNGGKQALETVQRLLPVLCQAHGLTPEQVVAIASHDGGKQALETVQRLLPVLCQAHGLTPEQVVAIASHDGGKQALETVQRLLPVLCQAHGLTPEQVVAIASNIGGKQALETVQALLPVLCQAHGLTPQQVVAIASNNGGKQALETVQRLLPVLCQAHGLTPEQVVAIASNIGGKQALETVQALLPVLCQAHGLTPQQVVAIASNGGGRPALESIVAQLSRPDPALAALTNDHLVALACLGGRPALDAVKKGLGDPISRSQLVKSELEEKKSELRHKLKYVPHEYIELIEIARNSTQDRILEMKVMEFFMKVYGYRGKHLGGSRKPDGAIYTVGSPIDYGVIVDTKAYSGGYNLPIGQADEMQRYVEENQTRNKHINPNEWWKVYPSSVTEFKFLFVSGHFKGNYKAQLTRLNHITNCNGAVLSVEELLIGGEMIKAGTLTLEEVRRKFNNGEINFAAD

SEQ ID NO: 12 - protein, 576 aa, artificial sequence
  CD22 CAR
MALPVTALLLPLALLLHAARPGGGGSCPYSNPSLCSGGGGSGGGGSQVQLQQSGPGLVKPSQTLSLTCAISGDSVSSNSAAWNWIRQSPSRGLEWLGRTYYRSKWYNDYAVSVKSRITINPDTSKNQFSLQLNSVTPEDTAVYYCAREVTGDLEDAFDIWGQGTMVTVSSGGGGSGGGGSGGGGSDIQMTQSPSSLSASVGDRVTITCRASQTIWSYLNWYQQRPGKAPNLLIYAASSLQSGVPSRFSGRGSGTDFTLTISSLQAEDFATYYCQQSYSIPQTFGQGTKLEIKSDPGSGGGGSCPYSNPSLCSGGGGSELPTQGTFSNVSTNVSPAKPTTTACPYSNPSLCAPTTTPAPRPPTPAPTIASQPLSLRPEACRPAAGGAVHTRGLDFACDIYIWAPLAGTCGVLLLSLVITLYCRRGRKKLLYIFKQPFMRPVQTTQEEDGCSCRFPEEEEGGCELRVKFSRSADAPAYQQGQNQLYNELNLGRREEYDVLDKRRGRDPEMGGKPRRKNPQEGLYNELQKDKMAEAYSEIGMKGERRRGKGHDGLYQGLSTATKDTYDALHMQALPPRE